European Patent Application EP 4 538 297 A1, published April 16, 2025. Title: GLYCOSYL-MODIFIED FUSION PROTEIN, NUCLEIC ACID MOLECULE, EXPRESSION VECTOR, HOST CELL AND APPLICATIONS THEREOF. Applicant: Kaimi Biomedicine (Chengdu) Co., Ltd. Application EP. The sequence listing filed with the application follows.

SEQUENCE LISTING (6 sequences)

SEQ ID NO: 1 - protein, 232 aa, Mus musculus
VDKKIVPRDCGCKPCICTVPEVSSVFIFPPKPKDVLTITLTPKVTCVVVDISKDDPEVQFSWFVDDVEVHTAQTQPREEQFNSTFRSVSELPIMHQDWLNGKEFKCRVNSAAFPAPIEKTISKTKGRPKAPQVYTIPPPKEQMAKDKVSLTCMITDFFPEDITVEWQWNGQPAENYKNTQPIMDTDGSYFVYSKLNVQKSNWEAGNTFTCSVLHEGLHNHHTEKSLSHSPGL

SEQ ID NO: 2 - protein, 232 aa, synthetic construct
VDKKIVPADCGCAPCICAVPEVSSVFIFPPKPKDVLTITLTPKVTCVVVDISKDDPEVQFSWFVDDVEVHTAQTQPREEQFNSTFRSVSELPIMHQDWLNGKEFKCRVNSAAFPAPIEKTISKTKGRPKAPQVYTIPPPKEQMAKDKVSLTCMITDFFPEDITVEWQWNGQPAENYKNTQPIMDTDGSYFVYSKLNVQKSNWEAGNTFTCSVLHEGLHNHHTEKSLSHSPGL

SEQ ID NO: 3 - protein, 232 aa, synthetic construct
VDKKIVPADCGCAPCICAVPEVSSVFIFPPKPKDVLTITLTPKVTCVVVDISKDDPEVQFSWFVDDVEVHTAQTQPREEQFNSTFRSVSELPIMHQDWLNGKEFKCRVNSAAFPLPEEKTISKTKGRPKAPQVYTIPPPKEQMAKDKVSLTCMITDFFPEDITVEWQWNGQPAENYKNTQPIMDTDGSYFVYSKLNVQKSNWEAGNTFTCSVLHEGLHNHHTEKSLSHSPGL

SEQ ID NO: 4 - protein, 592 aa, synthetic construct
KELKFVTLVFRHGDRSPIDTFPTDPIKESSWPQGFGQLTQLGMEQHYELGEYIRKRYRKFLNESYKHEQVYIRSTDVDRTLMSAMTNLAALFPPEGVSIWNPILLWQPIPVHTVPLSEDQLLYLPFRNCPRFQELESETLKSEEFQKRLHPYKDFIATLGKLSGLHGQDLFGIWSKVYDPLYCESVHNFTLPSWATEDTMTKLRELSELSLLSLYGIHKQKEKSRLQGGVLVNEILNHMKRATQIPSYKKLIMYSAHDTTVSGLQMALDVYNGLLPPYASCHLTELYFEKGEYFVEMYYRNETQHEPYPLMLPGCSPSCPLERFAELVGPVIPQDWSTECMTTNSHQGTEDSTDSRGGGSVDKKIVPADCGCAPCICAVPEVSSVFIFPPKPKDVLTITLTPKVTCVVVDISKDDPEVQFSWFVDDVEVHTAQTQPREEQFNSTFRSVSELPIMHQDWLNGKEFKCRVNSAAFPAPIEKTISKTKGRPKAPQVYTIPPPKEQMAKDKVSLTCMITDFFPEDITVEWQWNGQPAENYKNTQPIMDTDGSYFVYSKLNVQKSNWEAGNTFTCSVLHEGLHNHHTEKSLSHSPGL

SEQ ID NO: 5 - protein, 592 aa, synthetic construct
KELKFVTLVFRHGDRSPIDTFPTDPIKESSWPQGFGQLTQLGMEQHYELGEYIRKRYRKFLNESYKHEQVYIRSTDVDRTLMSAMTNLAALFPPEGVSIWNPILLWQPIPVHTVPLSEDQLLYLPFRNCPRFQELESETLKSEEFQKRLHPYKDFIATLGKLSGLHGQDLFGIWSKVYDPLYCESVHNFTLPSWATEDTMTKLRELSELSLLSLYGIHKQKEKSRLQGGVLVNEILNHMKRATQIPSYKKLIMYSAHDTTVSGLQMALDVYNGLLPPYASCHLTELYFEKGEYFVEMYYRNETQHEPYPLMLPGCSPSCPLERFAELVGPVIPQDWSTECMTTNSHQGTEDSTDSRGGGSVDKKIVPADCGCAPCICAVPEVSSVFIFPPKPKDVLTITLTPKVTCVVVDISKDDPEVQFSWFVDDVEVHTAQTQPREEQFNSTFRSVSELPIMHQDWLNGKEFKCRVNSAAFPLPEEKTISKTKGRPKAPQVYTIPPPKEQMAKDKVSLTCMITDFFPEDITVEWQWNGQPAENYKNTQPIMDTDGSYFVYSKLNVQKSNWEAGNTFTCSVLHEGLHNHHTEKSLSHSPGL

SEQ ID NO: 6 - protein, 597 aa, synthetic construct
KELKFVTLVFRHGDRSPIDTFPTDPIKESSWPQGFGQLTQLGMEQHYELGEYIRKRYRKFLNESYKHEQVYIRSTDVDRTLMSAMTNLAALFPPEGVSIWNPILLWQPIPVHTVPLSEDQLLYLPFRNCPRFQELESETLKSEEFQKRLHPYKDFIATLGKLSGLHGQDLFGIWSKVYDPLYCESVHNFTLPSWATEDTMTKLRELSELSLLSLYGIHKQKEKSRLQGGVLVNEILNHMKRATQIPSYKKLIMYSAHDTTVSGLQMALDVYNGLLPPYASCHLTELYFEKGEYFVEMYYRNETQHEPYPLMLPGCSPSCPLERFAELVGPVIPQDWSTECMTTNSHQGTEDSTDSRGGGSVDKRVEPKSCDKTHTCPPCPAPELLGGPSVFLFPPKPKDTLMISRTPEVTCVVVDVSHEDPEVKFNWYVDGVEVHNAKTKPREEQYNSTYRVVSVLTVLHQDWLNGKEYKCKVSNKALPAPIEKTISKAKGQPREPQVYTLPPSREEMTKNQVSLTCLVKGFYPSDIAVEWESNGQPENNYKTTPPVLDSDGSFFLYSKLTVDKSRWQQGNVFSCSVMHEALHNHYTQKSLSLSPGK